European Patent Application EP 4 541 885 A1, published April 23, 2025. Title: OPTIMIZED PHLOROGLUCINOL SYNTHASES. Applicant: COMPAGNIE GENERALE DES ETABLISSEMENTS MICHELIN. The sequence listing filed with the application follows.

SEQUENCE LISTING (76 sequences)

SEQ ID NO: 1 - protein, 390 aa, Tsukamurella pulmonis
MNTTEQQSVLPQQAWLGAPPAPPTSVAVIESLATSSPTQTYGQAESADRVAARFDDPRQAERIRRVYAKTRVTERHLAIDPLTPEFAEFSARPDTVRERMDLFFEHAAPLAIETARRALGDNAATDIGQLVFVTSTGFLAPGVDVAVIRALGLAPQTSRVVINFMGCAAAMNALRVSTDYVRAQPDRKSLMICLELSSVNAVFSGDPNDVVISSLFADGCGAAVIGASEVGHPLPSGQIVVRDTFTHLLDGAEDGIVLGVNANGITCELAESLPQYIVNGVAPVVDAVLDRNGLGREAVAHWAIHPGGPKIIESAAAALGLPDDASRLSWDVLAEHGNMLSVSLLFVLERLRAQVASDGADGAPSTGMAFSFAPGVTVEGFLFDVVTTGE

SEQ ID NO: 2 - protein, 390 aa, Synthetic construct
  VARIANT 271: note = X is any amino acid residue selected from the group consisting of arginine (R), histidine (H), lysine (K), glutamine (Q), valine (V), methionine (M), phenylalanine (F), leucine (L), tyrosine (Y), and proline (P)
MNTTEQQSVLPQQAWLGAPPAPPTSVAVIESLATXSPTQTYGQAEXADXVAARFDDPRQXERIRRVYAKTRVTERHLAIDPLTPEFAEFSXRXDTVRERMDLFFEHAAPLAIETARRALGDNXXTDIGXLVFVTSTGFLAPGVDVAVIRALGLXPQTSRVVINFMGCAAAMNALRXXTDYVRAQPDRKSLXICLELSSVNAVFSGDPNDVVISSLFADGCGAAVIGASEVGHPLPXGXIVVRDTFTHLLDGAEDGIVLGVNXNGITCXLXXSLPQYIVNGVAPVVDAVLXRNGLGREXVAHWAIHPGGPKIIESAAAALGLPDDASRLSWDVLAEHGNXLSVSLLFVLERLRAQVASDGADGAPSTGMAFSFAPGVTVEGFLFDVVTTGE

SEQ ID NO: 3 - protein, 390 aa, Synthetic construct
MNTTEQQSVLPQQAWLGAPPAPPTSVAVIESLATSSPTQTYGQAESADRVAARFDDPRQAERIRRVYAKTRVTERHLAIDPLTPEFAEFSARPDTVRERMDLFFEHAAPLAIETARRALGDNAPTDIGQLVFVTSTGFLAPGVDVAVIRALGLPPQTSRVVINFMGCAAAMNALRVATDYVRAQPDRKSLMICLELSSVNAVFSGDPNDVVISSLFADGCGAAVIGASEVGHPLPPGQIVVRDTFTHLLDGAEDGIVLGVNANGITCQLARSLPQYIVNGVAPVVDAVLDRNGLGREDVAHWAIHPGGPKIIESAAAALGLPDDASRLSWDVLAEHGNMLSVSLLFVLERLRAQVASDGADGAPSTGMAFSFAPGVTVEGFLFDVVTTGE

SEQ ID NO: 4 - protein, 390 aa, Synthetic construct
MNTTEQQSVLPQQAWLGAPPAPPTSVAVIESLATSSPTQTYGQAESADRVAARFDDPRQAERIRRVYAKTRVTERHLAIDPLTPEFAEFSARPDTVRERMDLFFEHAAPLAIETARRALGDNAPTDIGQLVFVTSTGFLAPGVDVAVIRALGLPPQTSRVVINFMGCAAAMNALRVATDYVRAQPDRKSLMICLELSSVNAVFSGDPNDVVISSLFADGCGAAVIGASEVGHPLPPGQIVVRDTFTHLLDGAEDGIVLGVNANGITCTLAKSLPQYIVNGVAPVVDAVLDRNGLGREDVAHWAIHPGGPKIIESAAAALGLPDDASRLSWDVLAEHGNMLSVSLLFVLERLRAQVASDGADGAPSTGMAFSFAPGVTVEGFLFDVVTTGE

SEQ ID NO: 5 - protein, 390 aa, Synthetic construct
MNTTEQQSVLPQQAWLGAPPAPPTSVAVIESLATSSPTQTYGQAESADRVAARFDDPRQAERIRRVYAKTRVTERHLAIDPLTPEFAEFSARPDTVRERMDLFFEHAAPLAIETARRALGDNAPTDIGQLVFVTSTGFLAPGVDVAVIRALGLPPQTSRVVINFMGCAAAMNALRVATDYVRAQPDRKSLMICLELSSVNAVFSGDPNDVVISSLFADGCGAAVIGASEVGHPLPPGQIVVRDTFTHLLDGAEDGIVLGVNANGITCSLSKSLPQYIVNGVAPVVDAVLDRNGLGREDVAHWAIHPGGPKIIESAAAALGLPDDASRLSWDVLAEHGNMLSVSLLFVLERLRAQVASDGADGAPSTGMAFSFAPGVTVEGFLFDVVTTGE

SEQ ID NO: 6 - protein, 390 aa, Synthetic construct
MNTTEQQSVLPQQAWLGAPPAPPTSVAVIESLATSSPTQTYGQAESADRVAARFDDPRQAERIRRVYAKTRVTERHLAIDPLTPEFAEFSARPDTVRERMDLFFEHAAPLAIETARRALGDNAPTDIGQLVFVTSTGFLAPGVDVAVIRALGLPPQTSRVVINFMGCAAAMNALRVATDYVRAQPDRKSLMICLELSSVNAVFSGDPNDVVISSLFADGCGAAVIGASEVGHPLPPGQIVVRDTFTHLLDGAEDGIVLGVNANGITCQLAKSLPQYIVNGVAPVVDAVLDRNGLGREDVAHWAIHPGGPKIIESAAAALGLPDDASRLSWDVLAEHGNMLSVSLLFVLERLRAQVASDGADGAPSTGMAFSFAPGVTVEGFLFDVVTTGE

SEQ ID NO: 7 - protein, 390 aa, Synthetic construct
MNTTEQQSVLPQQAWLGAPPAPPTSVAVIESLATSSPTQTYGQAESADRVAARFDDPRQAERIRRVYAKTRVTERHLAIDPLTPEFAEFSARPDTVRERMDLFFEHAAPLAIETARRALGDNAPTDIGQLVFVTSTGFLAPGVDVAVIRALGLPPQTSRVVINFMGCAAAMNALRVATDYVRAQPDRKSLMICLELSSVNAVFSGDPNDVVISSLFADGCGAAVIGASEVGHPLPPGQIVVRDTFTHLLDGAEDGIVLGVNANGITCSLARSLPQYIVNGVAPVVDAVLDRNGLGREDVAHWAIHPGGPKIIESAAAALGLPDDASRLSWDVLAEHGNMLSVSLLFVLERLRAQVASDGADGAPSTGMAFSFAPGVTVEGFLFDVVTTGE

SEQ ID NO: 8 - protein, 390 aa, Synthetic construct
MNTTEQQSVLPQQAWLGAPPAPPTSVAVIESLATSSPTQTYGQAESADRVAARFDDPRQAERIRRVYAKTRVTERHLAIDPLTPEFAEFSARPDTVRERMDLFFEHAAPLAIETARRALGDNAATDIGQLVFVTSTGFLAPGVDVAVIRALGLAPQTSRVVINFMGCAAAMNALRVSTDYVRAQPDRKSLMICLELSSVNAVFSGDPNDVVISSLFADGCGAAVIGASEVGHPLPSGQIVVRDTFTHLLDGAEDGIVLGVNANGITCQLAKSLPQYIVNGVAPVVDAVLDRNGLGREAVAHWAIHPGGPKIIESAAAALGLPDDASRLSWDVLAEHGNMLSVSLLFVLERLRAQVASDGADGAPSTGMAFSFAPGVTVEGFLFDVVTTGE

SEQ ID NO: 9 - protein, 390 aa, Synthetic construct
MNTTEQQSVLPQQAWLGAPPAPPTSVAVIESLATSSPTQTYGQAESADRVAARFDDPRQAERIRRVYAKTRVTERHLAIDPLTPEFAEFSARPDTVRERMDLFFEHAAPLAIETARRALGDNAATDIGQLVFVTSTGFLAPGVDVAVIRALGLAPQTSRVVINFMGCAAAMNALRVSTDYVRAQPDRKSLMICLELSSVNAVFSGDPNDVVISSLFADGCGAAVIGASEVGHPLPSGQIVVRDTFTHLLDGAEDGIVLGVNANGITCTLAKSLPQYIVNGVAPVVDAVLDRNGLGREAVAHWAIHPGGPKIIESAAAALGLPDDASRLSWDVLAEHGNMLSVSLLFVLERLRAQVASDGADGAPSTGMAFSFAPGVTVEGFLFDVVTTGE

SEQ ID NO: 10 - protein, 390 aa, Synthetic construct
MNTTEQQSVLPQQAWLGAPPAPPTSVAVIESLATSSPTQTYGQAESADRVAARFDDPRQAERIRRVYAKTRVTERHLAIDPLTPEFAEFSARPDTVRERMDLFFEHAAPLAIETARRALGDNAATDIGQLVFVTSTGFLAPGVDVAVIRALGLAPQTSRVVINFMGCAAAMNALRVSTDYVRAQPDRKSLMICLELSSVNAVFSGDPNDVVISSLFADGCGAAVIGASEVGHPLPSGQIVVRDTFTHLLDGAEDGIVLGVNANGITCTLARSLPQYIVNGVAPVVDAVLDRNGLGREAVAHWAIHPGGPKIIESAAAALGLPDDASRLSWDVLAEHGNMLSVSLLFVLERLRAQVASDGADGAPSTGMAFSFAPGVTVEGFLFDVVTTGE

SEQ ID NO: 11 - protein, 390 aa, Synthetic construct
MNTTEQQSVLPQQAWLGAPPAPPTSVAVIESLATSSPTQTYGQAESADRVAARFDDPRQAERIRRVYAKTRVTERHLAIDPLTPEFAEFSARPDTVRERMDLFFEHAAPLAIETARRALGDNAPTDIGQLVFVTSTGFLAPGVDVAVIRALGLPPQTSRVVINFMGCAAAMNALRVATDYVRAQPDRKSLMICLELSSVNAVFSGDPNDVVISSLFADGCGAAVIGASEVGHPLPPGQIVVRDTFTHLLDGAEDGIVLGVNANGITCQLSKSLPQYIVNGVAPVVDAVLDRNGLGREDVAHWAIHPGGPKIIESAAAALGLPDDASRLSWDVLAEHGNMLSVSLLFVLERLRAQVASDGADGAPSTGMAFSFAPGVTVEGFLFDVVTTGE

SEQ ID NO: 12 - protein, 390 aa, Synthetic construct
MNTTEQQSVLPQQAWLGAPPAPPTSVAVIESLATSSPTQTYGQAESADRVAARFDDPRQAERIRRVYAKTRVTERHLAIDPLTPEFAEFSARPDTVRERMDLFFEHAAPLAIETARRALGDNAPTDIGQLVFVTSTGFLAPGVDVAVIRALGLPPQTSRVVINFMGCAAAMNALRVATDYVRAQPDRKSLMICLELSSVNAVFSGDPNDVVISSLFADGCGAAVIGASEVGHPLPPGQIVVRDTFTHLLDGAEDGIVLGVNANGITCTLSRSLPQYIVNGVAPVVDAVLDRNGLGREDVAHWAIHPGGPKIIESAAAALGLPDDASRLSWDVLAEHGNMLSVSLLFVLERLRAQVASDGADGAPSTGMAFSFAPGVTVEGFLFDVVTTGE

SEQ ID NO: 13 - protein, 390 aa, Synthetic construct
MNTTEQQSVLPQQAWLGAPPAPPTSVAVIESLATSSPTQTYGQAESADRVAARFDDPRQAERIRRVYAKTRVTERHLAIDPLTPEFAEFSARPDTVRERMDLFFEHAAPLAIETARRALGDNAPTDIGQLVFVTSTGFLAPGVDVAVIRALGLPPQTSRVVINFMGCAAAMNALRVATDYVRAQPDRKSLMICLELSSVNAVFSGDPNDVVISSLFADGCGAAVIGASEVGHPLPPGQIVVRDTFTHLLDGAEDGIVLGVNANGITCTLSVSLPQYIVNGVAPVVDAVLDRNGLGREDVAHWAIHPGGPKIIESAAAALGLPDDASRLSWDVLAEHGNMLSVSLLFVLERLRAQVASDGADGAPSTGMAFSFAPGVTVEGFLFDVVTTGE

SEQ ID NO: 14 - protein, 390 aa, Synthetic construct
MNTTEQQSVLPQQAWLGAPPAPPTSVAVIESLATSSPTQTYGQAESADRVAARFDDPRQAERIRRVYAKTRVTERHLAIDPLTPEFAEFSARPDTVRERMDLFFEHAAPLAIETARRALGDNAPTDIGQLVFVTSTGFLAPGVDVAVIRALGLPPQTSRVVINFMGCAAAMNALRVATDYVRAQPDRKSLMICLELSSVNAVFSGDPNDVVISSLFADGCGAAVIGASEVGHPLPPGQIVVRDTFTHLLDGAEDGIVLGVNANGITCSLAKSLPQYIVNGVAPVVDAVLDRNGLGREDVAHWAIHPGGPKIIESAAAALGLPDDASRLSWDVLAEHGNMLSVSLLFVLERLRAQVASDGADGAPSTGMAFSFAPGVTVEGFLFDVVTTGE

SEQ ID NO: 15 - protein, 390 aa, Synthetic construct
MNTTEQQSVLPQQAWLGAPPAPPTSVAVIESLATSSPTQTYGQAESADRVAARFDDPRQAERIRRVYAKTRVTERHLAIDPLTPEFAEFSARPDTVRERMDLFFEHAAPLAIETARRALGDNAATDIGMLVFVTSTGFLAPGVDVAVIRALGLAPQTSRVVINFMGCAAAMNALRISTDYVRAQPDRKSLMICLELSSVNAVFSGDPNDVVISSLFADGCGAAVIGASEVGHPLPSGQIVVRDTFTHLLDGAEDGIVLGVNANGITCELAESLPQYIVNGVAPVVDAVLDRNGLGREAVAHWAIHPGGPKIIESAAAALGLPDDASRLSWDVLAEHGNMLSVSLLFVLERLRAQVASDGADGAPSTGMAFSFAPGVTVEGFLFDVVTTGE

SEQ ID NO: 16 - protein, 390 aa, Synthetic construct
MNTTEQQSVLPQQAWLGAPPAPPTSVAVIESLATSSPTQTYGQAESADRVAARFDDPRQAERIRRVYAKTRVTERHLAIDPLTPEFAEFSARPDTVRERMDLFFEHAAPLAIETARRALGDNAATDIGQLVFVTSTGFLAPGVDVAVIRALGLAPQTSRVVINFMGCAAAMNALRVSTDYVRAQPDRKSLMICLELSSVNAVFSGDPNDVVISSLFADGCGAAVIGASEVGHPLPSGQIVVRDTFTHLLDGAEDGIVLGVNANGITCQLARSLPQYIVNGVAPVVDAVLDRNGLGREAVAHWAIHPGGPKIIESAAAALGLPDDASRLSWDVLAEHGNMLSVSLLFVLERLRAQVASDGADGAPSTGMAFSFAPGVTVEGFLFDVVTTGE

SEQ ID NO: 17 - protein, 390 aa, Synthetic construct
MNTTEQQSVLPQQAWLGAPPAPPTSVAVIESLATSSPTQTYGQAESADRVAARFDDPRQAERIRRVYAKTRVTERHLAIDPLTPEFAEFSARPDTVRERMDLFFEHAAPLAIETARRALGDNAPTDIGQLVFVTSTGFLAPGVDVAVIRALGLPPQTSRVVINFMGCAAAMNALRVATDYVRAQPDRKSLMICLELSSVNAVFSGDPNDVVISSLFADGCGAAVIGASEVGHPLPPGQIVVRDTFTHLLDGAEDGIVLGVNANGITCQLSRSLPQYIVNGVAPVVDAVLDRNGLGREDVAHWAIHPGGPKIIESAAAALGLPDDASRLSWDVLAEHGNMLSVSLLFVLERLRAQVASDGADGAPSTGMAFSFAPGVTVEGFLFDVVTTGE

SEQ ID NO: 18 - protein, 390 aa, Synthetic construct
MNTTEQQSVLPQQAWLGAPPAPPTSVAVIESLATSSPTQTYGQAESADRVAARFDDPRQAERIRRVYAKTRVTERHLAIDPLTPEFAEFSARPDTVRERMDLFFEHAAPLAIETARRALGDNAPTDIGQLVFVTSTGFLAPGVDVAVIRALGLPPQTSRVVINFMGCAAAMNALRVATDYVRAQPDRKSLMICLELSSVNAVFSGDPNDVVISSLFADGCGAAVIGASEVGHPLPPGQIVVRDTFTHLLDGAEDGIVLGVNANGITCSLSRSLPQYIVNGVAPVVDAVLDRNGLGREDVAHWAIHPGGPKIIESAAAALGLPDDASRLSWDVLAEHGNMLSVSLLFVLERLRAQVASDGADGAPSTGMAFSFAPGVTVEGFLFDVVTTGE

SEQ ID NO: 19 - protein, 390 aa, Synthetic construct
MNTTEQQSVLPQQAWLGAPPAPPTSVAVIESLATSSPTQTYGQAESADRVAARFDDPRQAERIRRVYAKTRVTERHLAIDPLTPEFAEFSARPDTVRERMDLFFEHAAPLAIETARRALGDNAATDIGQLVFVTSTGFLAPGVDVAVIRALGLAPQTSRVVINFMGCAAAMNALRVSTDYVRAQPDRKSLMICLELSSVNAVFSGDPNDVVISSLFADGCGAAVIGASEVGHPLPSGQIVVRDTFTHLLDGAEDGIVLGVNANGITCELAKSLPQYIVNGVAPVVDAVLDRNGLGREAVAHWAIHPGGPKIIESAAAALGLPDDASRLSWDVLAEHGNMLSVSLLFVLERLRAQVASDGADGAPSTGMAFSFAPGVTVEGFLFDVVTTGE

SEQ ID NO: 20 - protein, 390 aa, Synthetic construct
MNTTEQQSVLPQQAWLGAPPAPPTSVAVIESLATGSPTQTYGQAESADRVAARFDDPRQRERIRRVYAKTRVTERHLAIDPLTPEFAEFSRRPDTVRERMDLFFEHAAPLAIETARRALGDNSPTDIGQLVFVTSTGFLAPGVDVAVIRALGLPPQTSRVVINFMGCAAAMNALRVATDYVRAQPDRKSLMICLELSSVNAVFSGDPNDVVISSLFADGCGAAVIGASEVGHPLPPGQIVVRDTFTHLLDGAEDGIVLGVNANGITCELSESLPQYIVNGVAPVVDAVLDRNGLGREDVAHWAIHPGGPKIIESAAAALGLPDDASRLSWDVLAEHGNMLSVSLLFVLERLRAQVASDGADGAPSTGMAFSFAPGVTVEGFLFDVVTTGE

SEQ ID NO: 21 - protein, 390 aa, Synthetic construct
MNTTEQQSVLPQQAWLGAPPAPPTSVAVIESLATSSPTQTYGQAESADRVAARFDDPRQAERIRRVYAKTRVTERHLAIDPLTPEFAEFSARPDTVRERMDLFFEHAAPLAIETARRALGDNAATDIGQLVFVTSTGFLAPGVDVAVIRALGLAPQTSRVVINFMGCAAAMNALRVSTDYVRAQPDRKSLMICLELSSVNAVFSGDPNDVVISSLFADGCGAAVIGASEVGHPLPSGQIVVRDTFTHLLDGAEDGIVLGVNANGITCSLAKSLPQYIVNGVAPVVDAVLDRNGLGREAVAHWAIHPGGPKIIESAAAALGLPDDASRLSWDVLAEHGNMLSVSLLFVLERLRAQVASDGADGAPSTGMAFSFAPGVTVEGFLFDVVTTGE

SEQ ID NO: 22 - protein, 390 aa, Synthetic construct
MNTTEQQSVLPQQAWLGAPPAPPTSVAVIESLATSSPTQTYGQAESADRVAARFDDPRQAERIRRVYAKTRVTERHLAIDPLTPEFAEFSARCDTVRERMDLFFEHAAPLAIETARRALGDNAATDIGQLVFVTSTGFLAPGVDVAVIRALGLAPQTSRVVINFMGCAAAMNALRVSTDYVRAQPDRKSLMICLELSSVNAVFSGDPNDVVISSLFADGCGAAVIGASEVGHPLPSGQIVVRDTFTHLLDGAEDGIVLGVNCNGITCELAESLPQYIVNGVAPVVDAVLDRNGLGREAVAHWAIHPGGPKIIESAAAALGLPDDASRLSWDVLAEHGNMLSVSLLFVLERLRAQVASDGADGAPSTGMAFSFAPGVTVEGFLFDVVTTGE

SEQ ID NO: 23 - protein, 390 aa, Synthetic construct
MNTTEQQSVLPQQAWLGAPPAPPTSVAVIESLATSSPTQTYGQAESADRVAARFDDPRQAERIRRVYAKTRVTERHLAIDPLTPEFAEFSARPDTVRERMDLFFEHAAPLAIETARRALGDNAATDIGQLVFVTSTGFLAPGVDVAVIRALGLAPQTSRVVINFMGCAAAMNALRVSTDYVRAQPDRKSLMICLELSSVNAVFSGDPNDVVISSLFADGCGAAVIGASEVGHPLPSGQIVVRDTFTHLLDGAEDGIVLGVNANGITCTLAVSLPQYIVNGVAPVVDAVLDRNGLGREAVAHWAIHPGGPKIIESAAAALGLPDDASRLSWDVLAEHGNMLSVSLLFVLERLRAQVASDGADGAPSTGMAFSFAPGVTVEGFLFDVVTTGE

SEQ ID NO: 24 - protein, 390 aa, Synthetic construct
MNTTEQQSVLPQQAWLGAPPAPPTSVAVIESLATSSPTQTYGQAESADRVAARFDDPRQAERIRRVYAKTRVTERHLAIDPLTPEFAEFSARPDTVRERMDLFFEHAAPLAIETARRALGDNAPTDIGQLVFVTSTGFLAPGVDVAVIRALGLPPQTSRVVINFMGCAAAMNALRVATDYVRAQPDRKSLMICLELSSVNAVFSGDPNDVVISSLFADGCGAAVIGASEVGHPLPPGQIVVRDTFTHLLDGAEDGIVLGVNANGITCTLSKSLPQYIVNGVAPVVDAVLDRNGLGREDVAHWAIHPGGPKIIESAAAALGLPDDASRLSWDVLAEHGNMLSVSLLFVLERLRAQVASDGADGAPSTGMAFSFAPGVTVEGFLFDVVTTGE

SEQ ID NO: 25 - protein, 390 aa, Synthetic construct
MNTTEQQSVLPQQAWLGAPPAPPTSVAVIESLATSSPTQTYGQAESADRVAARFDDPRQAERIRRVYAKTRVTERHLAIDPLTPEFAEFSARPDTVRERMDLFFEHAAPLAIETARRALGDNAATDIGQLVFVTSTGFLAPGVDVAVIRALGLAPQTSRVVINFMGCAAAMNALRVSTDYVRAQPDRKSLMICLELSSVNAVFSGDPNDVVISSLFADGCGAAVIGASEVGHPLPSGQIVVRDTFTHLLDGAEDGIVLGVNANGITCELARSLPQYIVNGVAPVVDAVLDRNGLGREAVAHWAIHPGGPKIIESAAAALGLPDDASRLSWDVLAEHGNMLSVSLLFVLERLRAQVASDGADGAPSTGMAFSFAPGVTVEGFLFDVVTTGE

SEQ ID NO: 26 - protein, 390 aa, Synthetic construct
MNTTEQQSVLPQQAWLGAPPAPPTSVAVIESLATGSPTQTYGQAEAADRVAARFDDPRQRERIRRVYAKTRVTERHLAIDPLTPEFAEFSRRPDTVRERMDLFFEHAAPLAIETARRALGDNSPTDIGQLVFVTSTGFLAPGVDVAVIRALGLPPQTSRVVINFMGCAAAMNALRVATDYVRAQPDRKSLVICLELSSVNAVFSGDPNDVVISSLFADGCGAAVIGASEVGHPLPPGKIVVRDTFTHLLDGAEDGIVLGVNANGITCELSESLPQYIVNGVAPVVDAVLARNGLGREDVAHWAIHPGGPKIIESAAAALGLPDDASRLSWDVLAEHGNMLSVSLLFVLERLRAQVASDGADGAPSTGMAFSFAPGVTVEGFLFDVVTTGE

SEQ ID NO: 27 - protein, 390 aa, Synthetic construct
MNTTEQQSVLPQQAWLGAPPAPPTSVAVIESLATSSPTQTYGQAESADAVAARFDDPRQAERIRRVYAKTRVTERHLAIDPLTPEFAEFSARPDTVRERMDLFFEHAAPLAIETARRALGDNAATDIGQLVFVTSTGFLAPGVDVAVIRALGLAPQTSRVVINFMGCAAAMNALRVSTDYVRAQPDRKSLMICLELSSVNAVFSGDPNDVVISSLFADGCGAAVIGASEVGHPLPSGQIVVRDTFTHLLDGAEDGIVLGVNANGITCELAESLPQYIVNGVAPVVDAVLDRNGLGREAVAHWAIHPGGPKIIESAAAALGLPDDASRLSWDVLAEHGNMLSVSLLFVLERLRAQVASDGADGAPSTGMAFSFAPGVTVEGFLFDVVTTGE

SEQ ID NO: 28 - protein, 390 aa, Synthetic construct
MNTTEQQSVLPQQAWLGAPPAPPTSVAVIESLATSSPTQTYGQAESADRVAARFDDPRQAERIRRVYAKTRVTERHLAIDPLTPEFAEFSARPDTVRERMDLFFEHAAPLAIETARRALGDNAATDIGQLVFVTSTGFLAPGVDVAVIRALGLAPQTSRVVINFMGCAAAMNALRVSTDYVRAQPDRKSLMICLELSSVNAVFSGDPNDVVISSLFADGCGAAVIGASEVGHPLPSGQIVVRDTFTHLLDGAEDGIVLGVNANGITCELAESLPQYIVNGVAPVVDAVLDRNGLGREAVAHWAIHPGGPKIIESAAAALGLPDDASRLSWDVLAEHGNILSVSLLFVLERLRAQVASDGADGAPSTGMAFSFAPGVTVEGFLFDVVTTGE

SEQ ID NO: 29 - DNA, 598 bp, Saccharomyces cerevisiae
  source 1..598: mol_type = genomic DNA
tatcttaactgatagtttgatcaaaggggcaaaacgtaggggcaaacaaacggaaaaatcgtttctcaaattttctgatgccaagaactctaaccagtcttatctaaaaattgccttatgatccgtctctccggttacagcctgtgtaactgattaatcctgcctttctaatcaccattctaatgttttaattaagggattttgtcttcattaacggctttcgctcataaaaatgttatgacgttttgcccgcaggcgggaaaccatccacttcacgagactgatctcctctgccggaacaccgggcatctccaacttataagttggagaaataagagaatttcagattgagagaatgaaaaaaaaaaaaaaaaaaggcagaggagagcatagaaatggggttcactttttggtaaagctatagcatgcctatcacatataaatagagtgccagtagcgacttttttcacactcgaaatactcttactactgctctcttgttgtttttatcacttcttgtttcttcttggtaaatagaatatcaagctacaaaaagcatacaatcaactatcaactattaactatatcgtaatacaca

SEQ ID NO: 30 - DNA, 998 bp, Saccharomyces cerevisiae
  source 1..998: mol_type = genomic DNA
aaccagggcaaagcaaaataaaagaaacttaatacgttatgccgtaatgaagggctaccaaaaacgataatctcaactgtaaacaggtacaatgcggacccttttgccacaaaacatacatcattcattgccggaaaaagaaagaagtgaagacagcagtgcagccagccatgttgcgccaatctaattatagatgctggtgccctgaggatgtatctggagccagccatggcatcatgcgctaccgccggatgtaaaatccgacacgcaaaagaaaaccttcgaggttgcgcacttcgcccacccatgaaccacacggttagtccaaaaggggcagttcagattccagatgcgggaattagcttgctgccaccctcacctcactaacgctgcggtgtgcggatacttcatgctatttatagacgcgcgtgtcggaatcagcacgcgcaagaaccaaatgggaaaatcggaatgggtccagaactgctttgagtgctggctattggcgtctgatttccgttttgggaatcctttgccgcgcgcccctctcaaaactccgcacaagtcccagaaagcgggaaagaaataaaacgccaccaaaaaaaaaaataaaagccaatcctcgaagcgtgggtggtaggccctggattatcccgtacaagtatttctcaggagtaaaaaaaccgtttgttttggaattccccatttcgcggccacctacgccgctatctttgcaacaactatctgcgataactcagcaaattttgcatattcgtgttgcagtattgcgataatgggagtcttacttccaacataacggcagaaagaaatgtgagaaaattttgcatcctttgcctccgttcaagtatataaagtcggcatgcttgataatctttctttccatcctacattgttctaattattcttattctcctttattctttcctaacataccaagaaattaatcttctgtcattcgcttaaacactatatcaata

SEQ ID NO: 31 - DNA, 400 bp, Saccharomyces cerevisiae
  source 1..400: mol_type = genomic DNA
catagcttcaaaatgtttctactccttttttactcttccagattttctcggactccgcgcatcgccgtaccacttcaaaacacccaagcacagcatactaaatttcccctctttcttcctctagggtgtcgttaattacccgtactaaaggtttggaaaagaaaaaagagaccgcctcgtttctttttcttcgtcgaaaaaggcaataaaaatttttatcacgtttctttttcttgaaaatttttttttttgatttttttctctttcgatgacctcccattgatatttaagttaataaacggtcttcaatttctcaagtttcagtttcatttttcttgttctattacaactttttttacttcttgctcattagaaagaaagcatagcaatctaatctaag

SEQ ID NO: 32 - DNA, 300 bp, Saccharomyces cerevisiae
  source 1..300: mol_type = genomic DNA
gaagttttgttagaaaataaatcattttttaattgagcattcttattcctattttatttaaatagttttatgtattgttagctacatacaacagtttaaatcaaattttctttttcccaagtccaaaatggaggtttattttgatgacccgcatgcgattatgttttgaaagtataagactacatacatgtacatatatttaaacatgtaaacccgtccattatattgcttactttcttcttttttgccgttttgacttggacctctggtttgctatttccttacaatctttgctacaat

SEQ ID NO: 33 - DNA, 188 bp, Saccharomyces cerevisiae
  source 1..188: mol_type = genomic DNA
gcgaatttcttatgatttatgatttttattattaaataagttataaaaaaaataagtgtatacaaattttaaagtgactcttaggttttaaaacgaaaattcttattcttgagtaactctttcctgtaggtcaggttgctttctcaggtatagcatgaggtcgctcttattgaccacacctctaccgg

SEQ ID NO: 34 - protein, 7 aa, Synthetic construct
DYKDDDK

SEQ ID NO: 35 - protein, 8 aa, Synthetic construct
WSHPQFEK

SEQ ID NO: 36 - protein, 9 aa, Synthetic construct
AWAHPQPGG

SEQ ID NO: 37 - protein, 6 aa, Synthetic construct
QYPALT

SEQ ID NO: 38 - protein, 6 aa, Synthetic construct
EYMPME

SEQ ID NO: 39 - protein, 6 aa, Synthetic construct
EFMPME

SEQ ID NO: 40 - protein, 11 aa, Synthetic construct
MASMTGGQQMG

SEQ ID NO: 41 - protein, 14 aa, Synthetic construct
GKPIPNPLLGLDST

SEQ ID NO: 42 - protein, 10 aa, Synthetic construct
SSTSSDFRDR

SEQ ID NO: 43 - protein, 19 aa, Synthetic construct
KDHLIHNVHKEFHAHAHNK

SEQ ID NO: 44 - protein, 6 aa, Synthetic construct
DTYRYI

SEQ ID NO: 45 - protein, 6 aa, Synthetic construct
TDFYLK

SEQ ID NO: 46 - DNA, 1173 bp, Tsukamurella pulmonis
  source 1..1173: mol_type = genomic DNA
atgaataccactgaacaacaatcagtcttgcctcaacaagcttggctgggagcaccaccagcccctccaactagcgttgcagtcatagaatcactggctacatcaagccccactcaaacctatggccaagctgaatccgctgatcgtgttgccgcgagatttgatgaccctagacaggctgaacgtattagaagggtttacgctaaaactcgtgttacggaaaggcatttagccattgatccattgactcctgagtttgctgaatttagcgcaaggcctgatacagttagggaaagaatggatttattttttgaacacgcagcacccttagctatagaaacagcaagaagagccctaggcgataatgcggccactgatattggtcagctagtttttgtgacatctacgggctttcttgcacctggtgtagatgttgccgttatcagagccttaggtctagcgcctcaaacctccagagttgttattaatttcatgggatgtgccgctgcaatgaatgccttgagagttagtaccgattatgtgagagcacaacctgatagaaagtcactgatgatttgcttagaattgagttccgtcaatgccgtatttagcggtgaccctaacgatgttgtcattagttcattgttcgctgatggttgcggtgcagctgtaataggtgcttccgaagtcggccatccattgccttctggccagatcgttgtaagggatacgtttactcatttgttagatggtgcggaagatgggatagtgctgggcgtcaacgcaaatgggatcacttgtgaattagcagaaagccttccacagtacattgtcaacggggtagctcccgtagtcgacgcagttttggacaggaacgggttggggagggaggcagttgcacattgggctatccatcctggaggtcctaaaataatagaatcagcagcagctgctttaggtctacccgatgatgcatctcgtttgtcatgggatgtcttagctgagcatggaaatatgttgtctgtatctctgctgtttgttttagagagattaagggcccaagttgcgagcgatggtgcggatggtgctccttccactgggatggcattttcatttgcacccggtgtgactgtagaagggttcctgtttgacgtggtaactacaggcgagtag

SEQ ID NO: 47 - DNA, 1173 bp, Synthetic construct
  source 1..1173: mol_type = other DNA
atgaataccactgaacaacaatcagtcttgcctcaacaagcttggctgggagcaccaccagcccctccaactagcgttgcagtcatagaatcactggctacatcaagccccactcaaacctatggccaagctgaatccgctgatcgtgttgccgcgagatttgatgaccctagacaggctgaacgtattagaagggtttacgctaaaactcgtgttacggaaaggcatttagccattgatccattgactcctgagtttgctgaatttagcgcaaggcctgatacagttagggaaagaatggatttattttttgaacacgcagcacccttagctatagaaacagcaagaagagccctaggcgataatgcgcctactgatattggtcagctagtttttgtgacatctacgggctttcttgcacctggtgtagatgttgccgttatcagagccttaggtctacctcctcaaacctccagagttgttattaatttcatgggatgtgccgctgcaatgaatgccttgagagttgcaaccgattatgtgagagcacaacctgatagaaagtcactgatgatttgcttagaattgagttccgtcaatgccgtatttagcggtgaccctaacgatgttgtcattagttcattgttcgctgatggttgcggtgcagctgtaataggtgcttccgaagtcggccatccattgcctcctggccagatcgttgtaagggatacgtttactcatttgttagatggtgcggaagatgggatagtgctgggcgtcaacgcaaatgggatcacttgtcaattagcaagaagccttccacagtacattgtcaacggggtagctcccgtagtcgacgcagttttggacaggaacgggttggggagggaggatgttgcacattgggctatccatcctggaggtcctaaaataatagaatcagcagcagctgctttaggtctacccgatgatgcatctcgtttgtcatgggatgtcttagctgagcatggaaatatgttgtctgtatctctgctgtttgttttagagagattaagggcccaagttgcgagcgatggtgcggatggtgctccttccactgggatggcattttcatttgcacccggtgtgactgtagaagggttcctgtttgacgtggtaactacaggcgagtag

SEQ ID NO: 48 - DNA, 1173 bp, Synthetic construct
  source 1..1173: mol_type = other DNA
atgaataccactgaacaacaatcagtcttgcctcaacaagcttggctgggagcaccaccagcccctccaactagcgttgcagtcatagaatcactggctacatcaagccccactcaaacctatggccaagctgaatccgctgatcgtgttgccgcgagatttgatgaccctagacaggctgaacgtattagaagggtttacgctaaaactcgtgttacggaaaggcatttagccattgatccattgactcctgagtttgctgaatttagcgcaaggcctgatacagttagggaaagaatggatttattttttgaacacgcagcacccttagctatagaaacagcaagaagagccctaggcgataatgcgcctactgatattggtcagctagtttttgtgacatctacgggctttcttgcacctggtgtagatgttgccgttatcagagccttaggtctacctcctcaaacctccagagttgttattaatttcatgggatgtgccgctgcaatgaatgccttgagagttgcaaccgattatgtgagagcacaacctgatagaaagtcactgatgatttgcttagaattgagttccgtcaatgccgtatttagcggtgaccctaacgatgttgtcattagttcattgttcgctgatggttgcggtgcagctgtaataggtgcttccgaagtcggccatccattgcctcctggccagatcgttgtaagggatacgtttactcatttgttagatggtgcggaagatgggatagtgctgggcgtcaacgcaaatgggatcacttgtactttagcaaaaagccttccacagtacattgtcaacggggtagctcccgtagtcgacgcagttttggacaggaacgggttggggagggaggatgttgcacattgggctatccatcctggaggtcctaaaataatagaatcagcagcagctgctttaggtctacccgatgatgcatctcgtttgtcatgggatgtcttagctgagcatggaaatatgttgtctgtatctctgctgtttgttttagagagattaagggcccaagttgcgagcgatggtgcggatggtgctccttccactgggatggcattttcatttgcacccggtgtgactgtagaagggttcctgtttgacgtggtaactacaggcgagtag

SEQ ID NO: 49 - DNA, 1173 bp, Synthetic construct
  source 1..1173: mol_type = other DNA
atgaataccactgaacaacaatcagtcttgcctcaacaagcttggctgggagcaccaccagcccctccaactagcgttgcagtcatagaatcactggctacatcaagccccactcaaacctatggccaagctgaatccgctgatcgtgttgccgcgagatttgatgaccctagacaggctgaacgtattagaagggtttacgctaaaactcgtgttacggaaaggcatttagccattgatccattgactcctgagtttgctgaatttagcgcaaggcctgatacagttagggaaagaatggatttattttttgaacacgcagcacccttagctatagaaacagcaagaagagccctaggcgataatgcgcctactgatattggtcagctagtttttgtgacatctacgggctttcttgcacctggtgtagatgttgccgttatcagagccttaggtctacctcctcaaacctccagagttgttattaatttcatgggatgtgccgctgcaatgaatgccttgagagttgcaaccgattatgtgagagcacaacctgatagaaagtcactgatgatttgcttagaattgagttccgtcaatgccgtatttagcggtgaccctaacgatgttgtcattagttcattgttcgctgatggttgcggtgcagctgtaataggtgcttccgaagtcggccatccattgcctcctggccagatcgttgtaagggatacgtttactcatttgttagatggtgcggaagatgggatagtgctgggcgtcaacgcaaatgggatcacttgttcattatcaaaaagccttccacagtacattgtcaacggggtagctcccgtagtcgacgcagttttggacaggaacgggttggggagggaggatgttgcacattgggctatccatcctggaggtcctaaaataatagaatcagcagcagctgctttaggtctacccgatgatgcatctcgtttgtcatgggatgtcttagctgagcatggaaatatgttgtctgtatctctgctgtttgttttagagagattaagggcccaagttgcgagcgatggtgcggatggtgctccttccactgggatggcattttcatttgcacccggtgtgactgtagaagggttcctgtttgacgtggtaactacaggcgagtag

SEQ ID NO: 50 - DNA, 1173 bp, Synthetic construct
  source 1..1173: mol_type = other DNA
atgaataccactgaacaacaatcagtcttgcctcaacaagcttggctgggagcaccaccagcccctccaactagcgttgcagtcatagaatcactggctacatcaagccccactcaaacctatggccaagctgaatccgctgatcgtgttgccgcgagatttgatgaccctagacaggctgaacgtattagaagggtttacgctaaaactcgtgttacggaaaggcatttagccattgatccattgactcctgagtttgctgaatttagcgcaaggcctgatacagttagggaaagaatggatttattttttgaacacgcagcacccttagctatagaaacagcaagaagagccctaggcgataatgcgcctactgatattggtcagctagtttttgtgacatctacgggctttcttgcacctggtgtagatgttgccgttatcagagccttaggtctacctcctcaaacctccagagttgttattaatttcatgggatgtgccgctgcaatgaatgccttgagagttgcaaccgattatgtgagagcacaacctgatagaaagtcactgatgatttgcttagaattgagttccgtcaatgccgtatttagcggtgaccctaacgatgttgtcattagttcattgttcgctgatggttgcggtgcagctgtaataggtgcttccgaagtcggccatccattgcctcctggccagatcgttgtaagggatacgtttactcatttgttagatggtgcggaagatgggatagtgctgggcgtcaacgcaaatgggatcacttgtcaattagcaaaaagccttccacagtacattgtcaacggggtagctcccgtagtcgacgcagttttggacaggaacgggttggggagggaggatgttgcacattgggctatccatcctggaggtcctaaaataatagaatcagcagcagctgctttaggtctacccgatgatgcatctcgtttgtcatgggatgtcttagctgagcatggaaatatgttgtctgtatctctgctgtttgttttagagagattaagggcccaagttgcgagcgatggtgcggatggtgctccttccactgggatggcattttcatttgcacccggtgtgactgtagaagggttcctgtttgacgtggtaactacaggcgagtag

SEQ ID NO: 51 - DNA, 1173 bp, Synthetic construct
  source 1..1173: mol_type = other DNA
atgaataccactgaacaacaatcagtcttgcctcaacaagcttggctgggagcaccaccagcccctccaactagcgttgcagtcatagaatcactggctacatcaagccccactcaaacctatggccaagctgaatccgctgatcgtgttgccgcgagatttgatgaccctagacaggctgaacgtattagaagggtttacgctaaaactcgtgttacggaaaggcatttagccattgatccattgactcctgagtttgctgaatttagcgcaaggcctgatacagttagggaaagaatggatttattttttgaacacgcagcacccttagctatagaaacagcaagaagagccctaggcgataatgcgcctactgatattggtcagctagtttttgtgacatctacgggctttcttgcacctggtgtagatgttgccgttatcagagccttaggtctacctcctcaaacctccagagttgttattaatttcatgggatgtgccgctgcaatgaatgccttgagagttgcaaccgattatgtgagagcacaacctgatagaaagtcactgatgatttgcttagaattgagttccgtcaatgccgtatttagcggtgaccctaacgatgttgtcattagttcattgttcgctgatggttgcggtgcagctgtaataggtgcttccgaagtcggccatccattgcctcctggccagatcgttgtaagggatacgtttactcatttgttagatggtgcggaagatgggatagtgctgggcgtcaacgcaaatgggatcacttgttcattagcaagaagccttccacagtacattgtcaacggggtagctcccgtagtcgacgcagttttggacaggaacgggttggggagggaggatgttgcacattgggctatccatcctggaggtcctaaaataatagaatcagcagcagctgctttaggtctacccgatgatgcatctcgtttgtcatgggatgtcttagctgagcatggaaatatgttgtctgtatctctgctgtttgttttagagagattaagggcccaagttgcgagcgatggtgcggatggtgctccttccactgggatggcattttcatttgcacccggtgtgactgtagaagggttcctgtttgacgtggtaactacaggcgagtag

SEQ ID NO: 52 - DNA, 1173 bp, Synthetic construct
  source 1..1173: mol_type = other DNA
atgaataccactgaacaacaatcagtcttgcctcaacaagcttggctgggagcaccaccagcccctccaactagcgttgcagtcatagaatcactggctacatcaagccccactcaaacctatggccaagctgaatccgctgatcgtgttgccgcgagatttgatgaccctagacaggctgaacgtattagaagggtttacgctaaaactcgtgttacggaaaggcatttagccattgatccattgactcctgagtttgctgaatttagcgcaaggcctgatacagttagggaaagaatggatttattttttgaacacgcagcacccttagctatagaaacagcaagaagagccctaggcgataatgcggccactgatattggtcagctagtttttgtgacatctacgggctttcttgcacctggtgtagatgttgccgttatcagagccttaggtctagcgcctcaaacctccagagttgttattaatttcatgggatgtgccgctgcaatgaatgccttgagagttagtaccgattatgtgagagcacaacctgatagaaagtcactgatgatttgcttagaattgagttccgtcaatgccgtatttagcggtgaccctaacgatgttgtcattagttcattgttcgctgatggttgcggtgcagctgtaataggtgcttccgaagtcggccatccattgccttctggccagatcgttgtaagggatacgtttactcatttgttagatggtgcggaagatgggatagtgctgggcgtcaacgcaaatgggatcacttgtcaattagcaaaaagccttccacagtacattgtcaacggggtagctcccgtagtcgacgcagttttggacaggaacgggttggggagggaggcagttgcacattgggctatccatcctggaggtcctaaaataatagaatcagcagcagctgctttaggtctacccgatgatgcatctcgtttgtcatgggatgtcttagctgagcatggaaatatgttgtctgtatctctgctgtttgttttagagagattaagggcccaagttgcgagcgatggtgcggatggtgctccttccactgggatggcattttcatttgcacccggtgtgactgtagaagggttcctgtttgacgtggtaactacaggcgagtag

SEQ ID NO: 53 - DNA, 1173 bp, Synthetic construct
  source 1..1173: mol_type = other DNA
atgaataccactgaacaacaatcagtcttgcctcaacaagcttggctgggagcaccaccagcccctccaactagcgttgcagtcatagaatcactggctacatcaagccccactcaaacctatggccaagctgaatccgctgatcgtgttgccgcgagatttgatgaccctagacaggctgaacgtattagaagggtttacgctaaaactcgtgttacggaaaggcatttagccattgatccattgactcctgagtttgctgaatttagcgcaaggcctgatacagttagggaaagaatggatttattttttgaacacgcagcacccttagctatagaaacagcaagaagagccctaggcgataatgcggccactgatattggtcagctagtttttgtgacatctacgggctttcttgcacctggtgtagatgttgccgttatcagagccttaggtctagcgcctcaaacctccagagttgttattaatttcatgggatgtgccgctgcaatgaatgccttgagagttagtaccgattatgtgagagcacaacctgatagaaagtcactgatgatttgcttagaattgagttccgtcaatgccgtatttagcggtgaccctaacgatgttgtcattagttcattgttcgctgatggttgcggtgcagctgtaataggtgcttccgaagtcggccatccattgccttctggccagatcgttgtaagggatacgtttactcatttgttagatggtgcggaagatgggatagtgctgggcgtcaacgcaaatgggatcacttgtactttagcaaaaagccttccacagtacattgtcaacggggtagctcccgtagtcgacgcagttttggacaggaacgggttggggagggaggcagttgcacattgggctatccatcctggaggtcctaaaataatagaatcagcagcagctgctttaggtctacccgatgatgcatctcgtttgtcatgggatgtcttagctgagcatggaaatatgttgtctgtatctctgctgtttgttttagagagattaagggcccaagttgcgagcgatggtgcggatggtgctccttccactgggatggcattttcatttgcacccggtgtgactgtagaagggttcctgtttgacgtggtaactacaggcgagtag

SEQ ID NO: 54 - DNA, 1173 bp, Synthetic construct
  source 1..1173: mol_type = other DNA
atgaataccactgaacaacaatcagtcttgcctcaacaagcttggctgggagcaccaccagcccctccaactagcgttgcagtcatagaatcactggctacatcaagccccactcaaacctatggccaagctgaatccgctgatcgtgttgccgcgagatttgatgaccctagacaggctgaacgtattagaagggtttacgctaaaactcgtgttacggaaaggcatttagccattgatccattgactcctgagtttgctgaatttagcgcaaggcctgatacagttagggaaagaatggatttattttttgaacacgcagcacccttagctatagaaacagcaagaagagccctaggcgataatgcggccactgatattggtcagctagtttttgtgacatctacgggctttcttgcacctggtgtagatgttgccgttatcagagccttaggtctagcgcctcaaacctccagagttgttattaatttcatgggatgtgccgctgcaatgaatgccttgagagttagtaccgattatgtgagagcacaacctgatagaaagtcactgatgatttgcttagaattgagttccgtcaatgccgtatttagcggtgaccctaacgatgttgtcattagttcattgttcgctgatggttgcggtgcagctgtaataggtgcttccgaagtcggccatccattgccttctggccagatcgttgtaagggatacgtttactcatttgttagatggtgcggaagatgggatagtgctgggcgtcaacgcaaatgggatcacttgtactttagcaagaagccttccacagtacattgtcaacggggtagctcccgtagtcgacgcagttttggacaggaacgggttggggagggaggcagttgcacattgggctatccatcctggaggtcctaaaataatagaatcagcagcagctgctttaggtctacccgatgatgcatctcgtttgtcatgggatgtcttagctgagcatggaaatatgttgtctgtatctctgctgtttgttttagagagattaagggcccaagttgcgagcgatggtgcggatggtgctccttccactgggatggcattttcatttgcacccggtgtgactgtagaagggttcctgtttgacgtggtaactacaggcgagtag

SEQ ID NO: 55 - DNA, 1173 bp, Synthetic construct
  source 1..1173: mol_type = other DNA
atgaataccactgaacaacaatcagtcttgcctcaacaagcttggctgggagcaccaccagcccctccaactagcgttgcagtcatagaatcactggctacatcaagccccactcaaacctatggccaagctgaatccgctgatcgtgttgccgcgagatttgatgaccctagacaggctgaacgtattagaagggtttacgctaaaactcgtgttacggaaaggcatttagccattgatccattgactcctgagtttgctgaatttagcgcaaggcctgatacagttagggaaagaatggatttattttttgaacacgcagcacccttagctatagaaacagcaagaagagccctaggcgataatgcgcctactgatattggtcagctagtttttgtgacatctacgggctttcttgcacctggtgtagatgttgccgttatcagagccttaggtctacctcctcaaacctccagagttgttattaatttcatgggatgtgccgctgcaatgaatgccttgagagttgcaaccgattatgtgagagcacaacctgatagaaagtcactgatgatttgcttagaattgagttccgtcaatgccgtatttagcggtgaccctaacgatgttgtcattagttcattgttcgctgatggttgcggtgcagctgtaataggtgcttccgaagtcggccatccattgcctcctggccagatcgttgtaagggatacgtttactcatttgttagatggtgcggaagatgggatagtgctgggcgtcaacgcaaatgggatcacttgtcaattatcaaaaagccttccacagtacattgtcaacggggtagctcccgtagtcgacgcagttttggacaggaacgggttggggagggaggatgttgcacattgggctatccatcctggaggtcctaaaataatagaatcagcagcagctgctttaggtctacccgatgatgcatctcgtttgtcatgggatgtcttagctgagcatggaaatatgttgtctgtatctctgctgtttgttttagagagattaagggcccaagttgcgagcgatggtgcggatggtgctccttccactgggatggcattttcatttgcacccggtgtgactgtagaagggttcctgtttgacgtggtaactacaggcgagtag

SEQ ID NO: 56 - DNA, 1173 bp, Synthetic construct
  source 1..1173: mol_type = other DNA
atgaataccactgaacaacaatcagtcttgcctcaacaagcttggctgggagcaccaccagcccctccaactagcgttgcagtcatagaatcactggctacatcaagccccactcaaacctatggccaagctgaatccgctgatcgtgttgccgcgagatttgatgaccctagacaggctgaacgtattagaagggtttacgctaaaactcgtgttacggaaaggcatttagccattgatccattgactcctgagtttgctgaatttagcgcaaggcctgatacagttagggaaagaatggatttattttttgaacacgcagcacccttagctatagaaacagcaagaagagccctaggcgataatgcgcctactgatattggtcagctagtttttgtgacatctacgggctttcttgcacctggtgtagatgttgccgttatcagagccttaggtctacctcctcaaacctccagagttgttattaatttcatgggatgtgccgctgcaatgaatgccttgagagttgcaaccgattatgtgagagcacaacctgatagaaagtcactgatgatttgcttagaattgagttccgtcaatgccgtatttagcggtgaccctaacgatgttgtcattagttcattgttcgctgatggttgcggtgcagctgtaataggtgcttccgaagtcggccatccattgcctcctggccagatcgttgtaagggatacgtttactcatttgttagatggtgcggaagatgggatagtgctgggcgtcaacgcaaatgggatcacttgtactttatcaagaagccttccacagtacattgtcaacggggtagctcccgtagtcgacgcagttttggacaggaacgggttggggagggaggatgttgcacattgggctatccatcctggaggtcctaaaataatagaatcagcagcagctgctttaggtctacccgatgatgcatctcgtttgtcatgggatgtcttagctgagcatggaaatatgttgtctgtatctctgctgtttgttttagagagattaagggcccaagttgcgagcgatggtgcggatggtgctccttccactgggatggcattttcatttgcacccggtgtgactgtagaagggttcctgtttgacgtggtaactacaggcgagtag

SEQ ID NO: 57 - DNA, 1173 bp, Synthetic construct
  source 1..1173: mol_type = other DNA
atgaataccactgaacaacaatcagtcttgcctcaacaagcttggctgggagcaccaccagcccctccaactagcgttgcagtcatagaatcactggctacatcaagccccactcaaacctatggccaagctgaatccgctgatcgtgttgccgcgagatttgatgaccctagacaggctgaacgtattagaagggtttacgctaaaactcgtgttacggaaaggcatttagccattgatccattgactcctgagtttgctgaatttagcgcaaggcctgatacagttagggaaagaatggatttattttttgaacacgcagcacccttagctatagaaacagcaagaagagccctaggcgataatgcgcctactgatattggtcagctagtttttgtgacatctacgggctttcttgcacctggtgtagatgttgccgttatcagagccttaggtctacctcctcaaacctccagagttgttattaatttcatgggatgtgccgctgcaatgaatgccttgagagttgcaaccgattatgtgagagcacaacctgatagaaagtcactgatgatttgcttagaattgagttccgtcaatgccgtatttagcggtgaccctaacgatgttgtcattagttcattgttcgctgatggttgcggtgcagctgtaataggtgcttccgaagtcggccatccattgcctcctggccagatcgttgtaagggatacgtttactcatttgttagatggtgcggaagatgggatagtgctgggcgtcaacgcaaatgggatcacttgtactttatcagttagccttccacagtacattgtcaacggggtagctcccgtagtcgacgcagttttggacaggaacgggttggggagggaggatgttgcacattgggctatccatcctggaggtcctaaaataatagaatcagcagcagctgctttaggtctacccgatgatgcatctcgtttgtcatgggatgtcttagctgagcatggaaatatgttgtctgtatctctgctgtttgttttagagagattaagggcccaagttgcgagcgatggtgcggatggtgctccttccactgggatggcattttcatttgcacccggtgtgactgtagaagggttcctgtttgacgtggtaactacaggcgagtag

SEQ ID NO: 58 - DNA, 1173 bp, Synthetic construct
  source 1..1173: mol_type = other DNA
atgaataccactgaacaacaatcagtcttgcctcaacaagcttggctgggagcaccaccagcccctccaactagcgttgcagtcatagaatcactggctacatcaagccccactcaaacctatggccaagctgaatccgctgatcgtgttgccgcgagatttgatgaccctagacaggctgaacgtattagaagggtttacgctaaaactcgtgttacggaaaggcatttagccattgatccattgactcctgagtttgctgaatttagcgcaaggcctgatacagttagggaaagaatggatttattttttgaacacgcagcacccttagctatagaaacagcaagaagagccctaggcgataatgcgcctactgatattggtcagctagtttttgtgacatctacgggctttcttgcacctggtgtagatgttgccgttatcagagccttaggtctacctcctcaaacctccagagttgttattaatttcatgggatgtgccgctgcaatgaatgccttgagagttgcaaccgattatgtgagagcacaacctgatagaaagtcactgatgatttgcttagaattgagttccgtcaatgccgtatttagcggtgaccctaacgatgttgtcattagttcattgttcgctgatggttgcggtgcagctgtaataggtgcttccgaagtcggccatccattgcctcctggccagatcgttgtaagggatacgtttactcatttgttagatggtgcggaagatgggatagtgctgggcgtcaacgcaaatgggatcacttgttcattagcaaaaagccttccacagtacattgtcaacggggtagctcccgtagtcgacgcagttttggacaggaacgggttggggagggaggatgttgcacattgggctatccatcctggaggtcctaaaataatagaatcagcagcagctgctttaggtctacccgatgatgcatctcgtttgtcatgggatgtcttagctgagcatggaaatatgttgtctgtatctctgctgtttgttttagagagattaagggcccaagttgcgagcgatggtgcggatggtgctccttccactgggatggcattttcatttgcacccggtgtgactgtagaagggttcctgtttgacgtggtaactacaggcgagtag

SEQ ID NO: 59 - DNA, 1173 bp, Synthetic construct
  source 1..1173: mol_type = other DNA
atgaataccactgaacaacaatcagtcttgcctcaacaagcttggctgggagcaccaccagcccctccaactagcgttgcagtcatagaatcactggctacatcaagccccactcaaacctatggccaagctgaatccgctgatcgtgttgccgcgagatttgatgaccctagacaggctgaacgtattagaagggtttacgctaaaactcgtgttacggaaaggcatttagccattgatccattgactcctgagtttgctgaatttagcgcaaggcctgatacagttagggaaagaatggatttattttttgaacacgcagcacccttagctatagaaacagcaagaagagccctaggcgataatgcggccactgatattggtatgctagtttttgtgacatctacgggctttcttgcacctggtgtagatgttgccgttatcagagccttaggtctagcgcctcaaacctccagagttgttattaatttcatgggatgtgccgctgcaatgaatgccttgagaattagtaccgattatgtgagagcacaacctgatagaaagtcactgatgatttgcttagaattgagttccgtcaatgccgtatttagcggtgaccctaacgatgttgtcattagttcattgttcgctgatggttgcggtgcagctgtaataggtgcttccgaagtcggccatccattgccttctggccagatcgttgtaagggatacgtttactcatttgttagatggtgcggaagatgggatagtgctgggcgtcaacgcaaatgggatcacttgtgaattagcagaaagccttccacagtacattgtcaacggggtagctcccgtagtcgacgcagttttggacaggaacgggttggggagggaggcagttgcacattgggctatccatcctggaggtcctaaaataatagaatcagcagcagctgctttaggtctacccgatgatgcatctcgtttgtcatgggatgtcttagctgagcatggaaatatgttgtctgtatctctgctgtttgttttagagagattaagggcccaagttgcgagcgatggtgcggatggtgctccttccactgggatggcattttcatttgcacccggtgtgactgtagaagggttcctgtttgacgtggtaactacaggcgagtag

SEQ ID NO: 60 - DNA, 1173 bp, Synthetic construct
  source 1..1173: mol_type = other DNA
atgaataccactgaacaacaatcagtcttgcctcaacaagcttggctgggagcaccaccagcccctccaactagcgttgcagtcatagaatcactggctacatcaagccccactcaaacctatggccaagctgaatccgctgatcgtgttgccgcgagatttgatgaccctagacaggctgaacgtattagaagggtttacgctaaaactcgtgttacggaaaggcatttagccattgatccattgactcctgagtttgctgaatttagcgcaaggcctgatacagttagggaaagaatggatttattttttgaacacgcagcacccttagctatagaaacagcaagaagagccctaggcgataatgcggccactgatattggtcagctagtttttgtgacatctacgggctttcttgcacctggtgtagatgttgccgttatcagagccttaggtctagcgcctcaaacctccagagttgttattaatttcatgggatgtgccgctgcaatgaatgccttgagagttagtaccgattatgtgagagcacaacctgatagaaagtcactgatgatttgcttagaattgagttccgtcaatgccgtatttagcggtgaccctaacgatgttgtcattagttcattgttcgctgatggttgcggtgcagctgtaataggtgcttccgaagtcggccatccattgccttctggccagatcgttgtaagggatacgtttactcatttgttagatggtgcggaagatgggatagtgctgggcgtcaacgcaaatgggatcacttgtcaattagcaagaagccttccacagtacattgtcaacggggtagctcccgtagtcgacgcagttttggacaggaacgggttggggagggaggcagttgcacattgggctatccatcctggaggtcctaaaataatagaatcagcagcagctgctttaggtctacccgatgatgcatctcgtttgtcatgggatgtcttagctgagcatggaaatatgttgtctgtatctctgctgtttgttttagagagattaagggcccaagttgcgagcgatggtgcggatggtgctccttccactgggatggcattttcatttgcacccggtgtgactgtagaagggttcctgtttgacgtggtaactacaggcgagtag

SEQ ID NO: 61 - DNA, 1173 bp, Synthetic construct
  source 1..1173: mol_type = other DNA
atgaataccactgaacaacaatcagtcttgcctcaacaagcttggctgggagcaccaccagcccctccaactagcgttgcagtcatagaatcactggctacatcaagccccactcaaacctatggccaagctgaatccgctgatcgtgttgccgcgagatttgatgaccctagacaggctgaacgtattagaagggtttacgctaaaactcgtgttacggaaaggcatttagccattgatccattgactcctgagtttgctgaatttagcgcaaggcctgatacagttagggaaagaatggatttattttttgaacacgcagcacccttagctatagaaacagcaagaagagccctaggcgataatgcgcctactgatattggtcagctagtttttgtgacatctacgggctttcttgcacctggtgtagatgttgccgttatcagagccttaggtctacctcctcaaacctccagagttgttattaatttcatgggatgtgccgctgcaatgaatgccttgagagttgcaaccgattatgtgagagcacaacctgatagaaagtcactgatgatttgcttagaattgagttccgtcaatgccgtatttagcggtgaccctaacgatgttgtcattagttcattgttcgctgatggttgcggtgcagctgtaataggtgcttccgaagtcggccatccattgcctcctggccagatcgttgtaagggatacgtttactcatttgttagatggtgcggaagatgggatagtgctgggcgtcaacgcaaatgggatcacttgtcaattatcaagaagccttccacagtacattgtcaacggggtagctcccgtagtcgacgcagttttggacaggaacgggttggggagggaggatgttgcacattgggctatccatcctggaggtcctaaaataatagaatcagcagcagctgctttaggtctacccgatgatgcatctcgtttgtcatgggatgtcttagctgagcatggaaatatgttgtctgtatctctgctgtttgttttagagagattaagggcccaagttgcgagcgatggtgcggatggtgctccttccactgggatggcattttcatttgcacccggtgtgactgtagaagggttcctgtttgacgtggtaactacaggcgagtag

SEQ ID NO: 62 - DNA, 1173 bp, Synthetic construct
  source 1..1173: mol_type = other DNA
atgaataccactgaacaacaatcagtcttgcctcaacaagcttggctgggagcaccaccagcccctccaactagcgttgcagtcatagaatcactggctacatcaagccccactcaaacctatggccaagctgaatccgctgatcgtgttgccgcgagatttgatgaccctagacaggctgaacgtattagaagggtttacgctaaaactcgtgttacggaaaggcatttagccattgatccattgactcctgagtttgctgaatttagcgcaaggcctgatacagttagggaaagaatggatttattttttgaacacgcagcacccttagctatagaaacagcaagaagagccctaggcgataatgcgcctactgatattggtcagctagtttttgtgacatctacgggctttcttgcacctggtgtagatgttgccgttatcagagccttaggtctacctcctcaaacctccagagttgttattaatttcatgggatgtgccgctgcaatgaatgccttgagagttgcaaccgattatgtgagagcacaacctgatagaaagtcactgatgatttgcttagaattgagttccgtcaatgccgtatttagcggtgaccctaacgatgttgtcattagttcattgttcgctgatggttgcggtgcagctgtaataggtgcttccgaagtcggccatccattgcctcctggccagatcgttgtaagggatacgtttactcatttgttagatggtgcggaagatgggatagtgctgggcgtcaacgcaaatgggatcacttgttcattatcaagaagccttccacagtacattgtcaacggggtagctcccgtagtcgacgcagttttggacaggaacgggttggggagggaggatgttgcacattgggctatccatcctggaggtcctaaaataatagaatcagcagcagctgctttaggtctacccgatgatgcatctcgtttgtcatgggatgtcttagctgagcatggaaatatgttgtctgtatctctgctgtttgttttagagagattaagggcccaagttgcgagcgatggtgcggatggtgctccttccactgggatggcattttcatttgcacccggtgtgactgtagaagggttcctgtttgacgtggtaactacaggcgagtag

SEQ ID NO: 63 - DNA, 1173 bp, Synthetic construct
  source 1..1173: mol_type = other DNA
atgaataccactgaacaacaatcagtcttgcctcaacaagcttggctgggagcaccaccagcccctccaactagcgttgcagtcatagaatcactggctacatcaagccccactcaaacctatggccaagctgaatccgctgatcgtgttgccgcgagatttgatgaccctagacaggctgaacgtattagaagggtttacgctaaaactcgtgttacggaaaggcatttagccattgatccattgactcctgagtttgctgaatttagcgcaaggcctgatacagttagggaaagaatggatttattttttgaacacgcagcacccttagctatagaaacagcaagaagagccctaggcgataatgcggccactgatattggtcagctagtttttgtgacatctacgggctttcttgcacctggtgtagatgttgccgttatcagagccttaggtctagcgcctcaaacctccagagttgttattaatttcatgggatgtgccgctgcaatgaatgccttgagagttagtaccgattatgtgagagcacaacctgatagaaagtcactgatgatttgcttagaattgagttccgtcaatgccgtatttagcggtgaccctaacgatgttgtcattagttcattgttcgctgatggttgcggtgcagctgtaataggtgcttccgaagtcggccatccattgccttctggccagatcgttgtaagggatacgtttactcatttgttagatggtgcggaagatgggatagtgctgggcgtcaacgcaaatgggatcacttgtgaattagcaaaaagccttccacagtacattgtcaacggggtagctcccgtagtcgacgcagttttggacaggaacgggttggggagggaggcagttgcacattgggctatccatcctggaggtcctaaaataatagaatcagcagcagctgctttaggtctacccgatgatgcatctcgtttgtcatgggatgtcttagctgagcatggaaatatgttgtctgtatctctgctgtttgttttagagagattaagggcccaagttgcgagcgatggtgcggatggtgctccttccactgggatggcattttcatttgcacccggtgtgactgtagaagggttcctgtttgacgtggtaactacaggcgagtag

SEQ ID NO: 64 - DNA, 1173 bp, Synthetic construct
  source 1..1173: mol_type = other DNA
atgaataccactgaacaacaatcagtcttgcctcaacaagcttggctgggagcaccaccagcccctccaactagcgttgcagtcatagaatcactggctacaggtagccccactcaaacctatggccaagctgaatccgctgatcgtgttgccgcgagatttgatgaccctagacagagagaacgtattagaagggtttacgctaaaactcgtgttacggaaaggcatttagccattgatccattgactcctgagtttgctgaatttagcagaaggcctgatacagttagggaaagaatggatttattttttgaacacgcagcacccttagctatagaaacagcaagaagagccctaggcgataattcacctactgatattggtcagctagtttttgtgacatctacgggctttcttgcacctggtgtagatgttgccgttatcagagccttaggtctacctcctcaaacctccagagttgttattaatttcatgggatgtgccgctgcaatgaatgccttgagagttgcaaccgattatgtgagagcacaacctgatagaaagtcactgatgatttgcttagaattgagttccgtcaatgccgtatttagcggtgaccctaacgatgttgtcattagttcattgttcgctgatggttgcggtgcagctgtaataggtgcttccgaagtcggccatccattgcctcctggccagatcgttgtaagggatacgtttactcatttgttagatggtgcggaagatgggatagtgctgggcgtcaacgcaaatgggatcacttgtgaattatcagaaagccttccacagtacattgtcaacggggtagctcccgtagtcgacgcagttttggacaggaacgggttggggagggaggatgttgcacattgggctatccatcctggaggtcctaaaataatagaatcagcagcagctgctttaggtctacccgatgatgcatctcgtttgtcatgggatgtcttagctgagcatggaaatatgttgtctgtatctctgctgtttgttttagagagattaagggcccaagttgcgagcgatggtgcggatggtgctccttccactgggatggcattttcatttgcacccggtgtgactgtagaagggttcctgtttgacgtggtaactacaggcgagtag

SEQ ID NO: 65 - DNA, 1173 bp, Synthetic construct
  source 1..1173: mol_type = other DNA
atgaataccactgaacaacaatcagtcttgcctcaacaagcttggctgggagcaccaccagcccctccaactagcgttgcagtcatagaatcactggctacatcaagccccactcaaacctatggccaagctgaatccgctgatcgtgttgccgcgagatttgatgaccctagacaggctgaacgtattagaagggtttacgctaaaactcgtgttacggaaaggcatttagccattgatccattgactcctgagtttgctgaatttagcgcaaggcctgatacagttagggaaagaatggatttattttttgaacacgcagcacccttagctatagaaacagcaagaagagccctaggcgataatgcggccactgatattggtcagctagtttttgtgacatctacgggctttcttgcacctggtgtagatgttgccgttatcagagccttaggtctagcgcctcaaacctccagagttgttattaatttcatgggatgtgccgctgcaatgaatgccttgagagttagtaccgattatgtgagagcacaacctgatagaaagtcactgatgatttgcttagaattgagttccgtcaatgccgtatttagcggtgaccctaacgatgttgtcattagttcattgttcgctgatggttgcggtgcagctgtaataggtgcttccgaagtcggccatccattgccttctggccagatcgttgtaagggatacgtttactcatttgttagatggtgcggaagatgggatagtgctgggcgtcaacgcaaatgggatcacttgttcattagcaaaaagccttccacagtacattgtcaacggggtagctcccgtagtcgacgcagttttggacaggaacgggttggggagggaggcagttgcacattgggctatccatcctggaggtcctaaaataatagaatcagcagcagctgctttaggtctacccgatgatgcatctcgtttgtcatgggatgtcttagctgagcatggaaatatgttgtctgtatctctgctgtttgttttagagagattaagggcccaagttgcgagcgatggtgcggatggtgctccttccactgggatggcattttcatttgcacccggtgtgactgtagaagggttcctgtttgacgtggtaactacaggcgagtag

SEQ ID NO: 66 - DNA, 1173 bp, Synthetic construct
  source 1..1173: mol_type = other DNA
atgaataccactgaacaacaatcagtcttgcctcaacaagcttggctgggagcaccaccagcccctccaactagcgttgcagtcatagaatcactggctacatcaagccccactcaaacctatggccaagctgaatccgctgatcgtgttgccgcgagatttgatgaccctagacaggctgaacgtattagaagggtttacgctaaaactcgtgttacggaaaggcatttagccattgatccattgactcctgagtttgctgaatttagcgcaaggtgcgatacagttagggaaagaatggatttattttttgaacacgcagcacccttagctatagaaacagcaagaagagccctaggcgataatgcggccactgatattggtcagctagtttttgtgacatctacgggctttcttgcacctggtgtagatgttgccgttatcagagccttaggtctagcgcctcaaacctccagagttgttattaatttcatgggatgtgccgctgcaatgaatgccttgagagttagtaccgattatgtgagagcacaacctgatagaaagtcactgatgatttgcttagaattgagttccgtcaatgccgtatttagcggtgaccctaacgatgttgtcattagttcattgttcgctgatggttgcggtgcagctgtaataggtgcttccgaagtcggccatccattgccttctggccagatcgttgtaagggatacgtttactcatttgttagatggtgcggaagatgggatagtgctgggcgtcaactgcaatgggatcacttgtgaattagcagaaagccttccacagtacattgtcaacggggtagctcccgtagtcgacgcagttttggacaggaacgggttggggagggaggcagttgcacattgggctatccatcctggaggtcctaaaataatagaatcagcagcagctgctttaggtctacccgatgatgcatctcgtttgtcatgggatgtcttagctgagcatggaaatatgttgtctgtatctctgctgtttgttttagagagattaagggcccaagttgcgagcgatggtgcggatggtgctccttccactgggatggcattttcatttgcacccggtgtgactgtagaagggttcctgtttgacgtggtaactacaggcgagtag

SEQ ID NO: 67 - DNA, 1173 bp, Synthetic construct
  source 1..1173: mol_type = other DNA
atgaataccactgaacaacaatcagtcttgcctcaacaagcttggctgggagcaccaccagcccctccaactagcgttgcagtcatagaatcactggctacatcaagccccactcaaacctatggccaagctgaatccgctgatcgtgttgccgcgagatttgatgaccctagacaggctgaacgtattagaagggtttacgctaaaactcgtgttacggaaaggcatttagccattgatccattgactcctgagtttgctgaatttagcgcaaggcctgatacagttagggaaagaatggatttattttttgaacacgcagcacccttagctatagaaacagcaagaagagccctaggcgataatgcggccactgatattggtcagctagtttttgtgacatctacgggctttcttgcacctggtgtagatgttgccgttatcagagccttaggtctagcgcctcaaacctccagagttgttattaatttcatgggatgtgccgctgcaatgaatgccttgagagttagtaccgattatgtgagagcacaacctgatagaaagtcactgatgatttgcttagaattgagttccgtcaatgccgtatttagcggtgaccctaacgatgttgtcattagttcattgttcgctgatggttgcggtgcagctgtaataggtgcttccgaagtcggccatccattgccttctggccagatcgttgtaagggatacgtttactcatttgttagatggtgcggaagatgggatagtgctgggcgtcaacgcaaatgggatcacttgtactttagcagttagccttccacagtacattgtcaacggggtagctcccgtagtcgacgcagttttggacaggaacgggttggggagggaggcagttgcacattgggctatccatcctggaggtcctaaaataatagaatcagcagcagctgctttaggtctacccgatgatgcatctcgtttgtcatgggatgtcttagctgagcatggaaatatgttgtctgtatctctgctgtttgttttagagagattaagggcccaagttgcgagcgatggtgcggatggtgctccttccactgggatggcattttcatttgcacccggtgtgactgtagaagggttcctgtttgacgtggtaactacaggcgagtag

SEQ ID NO: 68 - DNA, 1173 bp, Synthetic construct
  source 1..1173: mol_type = other DNA
atgaataccactgaacaacaatcagtcttgcctcaacaagcttggctgggagcaccaccagcccctccaactagcgttgcagtcatagaatcactggctacatcaagccccactcaaacctatggccaagctgaatccgctgatcgtgttgccgcgagatttgatgaccctagacaggctgaacgtattagaagggtttacgctaaaactcgtgttacggaaaggcatttagccattgatccattgactcctgagtttgctgaatttagcgcaaggcctgatacagttagggaaagaatggatttattttttgaacacgcagcacccttagctatagaaacagcaagaagagccctaggcgataatgcgcctactgatattggtcagctagtttttgtgacatctacgggctttcttgcacctggtgtagatgttgccgttatcagagccttaggtctacctcctcaaacctccagagttgttattaatttcatgggatgtgccgctgcaatgaatgccttgagagttgcaaccgattatgtgagagcacaacctgatagaaagtcactgatgatttgcttagaattgagttccgtcaatgccgtatttagcggtgaccctaacgatgttgtcattagttcattgttcgctgatggttgcggtgcagctgtaataggtgcttccgaagtcggccatccattgcctcctggccagatcgttgtaagggatacgtttactcatttgttagatggtgcggaagatgggatagtgctgggcgtcaacgcaaatgggatcacttgtactttatcaaaaagccttccacagtacattgtcaacggggtagctcccgtagtcgacgcagttttggacaggaacgggttggggagggaggatgttgcacattgggctatccatcctggaggtcctaaaataatagaatcagcagcagctgctttaggtctacccgatgatgcatctcgtttgtcatgggatgtcttagctgagcatggaaatatgttgtctgtatctctgctgtttgttttagagagattaagggcccaagttgcgagcgatggtgcggatggtgctccttccactgggatggcattttcatttgcacccggtgtgactgtagaagggttcctgtttgacgtggtaactacaggcgagtag

SEQ ID NO: 69 - DNA, 1173 bp, Synthetic construct
  source 1..1173: mol_type = other DNA
atgaataccactgaacaacaatcagtcttgcctcaacaagcttggctgggagcaccaccagcccctccaactagcgttgcagtcatagaatcactggctacatcaagccccactcaaacctatggccaagctgaatccgctgatcgtgttgccgcgagatttgatgaccctagacaggctgaacgtattagaagggtttacgctaaaactcgtgttacggaaaggcatttagccattgatccattgactcctgagtttgctgaatttagcgcaaggcctgatacagttagggaaagaatggatttattttttgaacacgcagcacccttagctatagaaacagcaagaagagccctaggcgataatgcggccactgatattggtcagctagtttttgtgacatctacgggctttcttgcacctggtgtagatgttgccgttatcagagccttaggtctagcgcctcaaacctccagagttgttattaatttcatgggatgtgccgctgcaatgaatgccttgagagttagtaccgattatgtgagagcacaacctgatagaaagtcactgatgatttgcttagaattgagttccgtcaatgccgtatttagcggtgaccctaacgatgttgtcattagttcattgttcgctgatggttgcggtgcagctgtaataggtgcttccgaagtcggccatccattgccttctggccagatcgttgtaagggatacgtttactcatttgttagatggtgcggaagatgggatagtgctgggcgtcaacgcaaatgggatcacttgtgaattagcaagaagccttccacagtacattgtcaacggggtagctcccgtagtcgacgcagttttggacaggaacgggttggggagggaggcagttgcacattgggctatccatcctggaggtcctaaaataatagaatcagcagcagctgctttaggtctacccgatgatgcatctcgtttgtcatgggatgtcttagctgagcatggaaatatgttgtctgtatctctgctgtttgttttagagagattaagggcccaagttgcgagcgatggtgcggatggtgctccttccactgggatggcattttcatttgcacccggtgtgactgtagaagggttcctgtttgacgtggtaactacaggcgagtag

SEQ ID NO: 70 - DNA, 1173 bp, Synthetic construct
  source 1..1173: mol_type = other DNA
atgaataccactgaacaacaatcagtcttgcctcaacaagcttggctgggagcaccaccagcccctccaactagcgttgcagtcatagaatcactggctacaggtagccccactcaaacctatggccaagctgaagcagctgatcgtgttgccgcgagatttgatgaccctagacagagagaacgtattagaagggtttacgctaaaactcgtgttacggaaaggcatttagccattgatccattgactcctgagtttgctgaatttagcagaaggcctgatacagttagggaaagaatggatttattttttgaacacgcagcacccttagctatagaaacagcaagaagagccctaggcgataattcacctactgatattggtcagctagtttttgtgacatctacgggctttcttgcacctggtgtagatgttgccgttatcagagccttaggtctacctcctcaaacctccagagttgttattaatttcatgggatgtgccgctgcaatgaatgccttgagagttgcaaccgattatgtgagagcacaacctgatagaaagtcactggttatttgcttagaattgagttccgtcaatgccgtatttagcggtgaccctaacgatgttgtcattagttcattgttcgctgatggttgcggtgcagctgtaataggtgcttccgaagtcggccatccattgcctcctggcaaaatcgttgtaagggatacgtttactcatttgttagatggtgcggaagatgggatagtgctgggcgtcaacgcaaatgggatcacttgtgaattatcagaaagccttccacagtacattgtcaacggggtagctcccgtagtcgacgcagttttggcaaggaacgggttggggagggaggatgttgcacattgggctatccatcctggaggtcctaaaataatagaatcagcagcagctgctttaggtctacccgatgatgcatctcgtttgtcatgggatgtcttagctgagcatggaaatatgttgtctgtatctctgctgtttgttttagagagattaagggcccaagttgcgagcgatggtgcggatggtgctccttccactgggatggcattttcatttgcacccggtgtgactgtagaagggttcctgtttgacgtggtaactacaggcgagtag

SEQ ID NO: 71 - DNA, 1173 bp, Synthetic construct
  source 1..1173: mol_type = other DNA
atgaataccactgaacaacaatcagtcttgcctcaacaagcttggctgggagcaccaccagcccctccaactagcgttgcagtcatagaatcactggctacatcaagccccactcaaacctatggccaagctgaatccgctgatgcagttgccgcgagatttgatgaccctagacaggctgaacgtattagaagggtttacgctaaaactcgtgttacggaaaggcatttagccattgatccattgactcctgagtttgctgaatttagcgcaaggcctgatacagttagggaaagaatggatttattttttgaacacgcagcacccttagctatagaaacagcaagaagagccctaggcgataatgcggccactgatattggtcagctagtttttgtgacatctacgggctttcttgcacctggtgtagatgttgccgttatcagagccttaggtctagcgcctcaaacctccagagttgttattaatttcatgggatgtgccgctgcaatgaatgccttgagagttagtaccgattatgtgagagcacaacctgatagaaagtcactgatgatttgcttagaattgagttccgtcaatgccgtatttagcggtgaccctaacgatgttgtcattagttcattgttcgctgatggttgcggtgcagctgtaataggtgcttccgaagtcggccatccattgccttctggccagatcgttgtaagggatacgtttactcatttgttagatggtgcggaagatgggatagtgctgggcgtcaacgcaaatgggatcacttgtgaattagcagaaagccttccacagtacattgtcaacggggtagctcccgtagtcgacgcagttttggacaggaacgggttggggagggaggcagttgcacattgggctatccatcctggaggtcctaaaataatagaatcagcagcagctgctttaggtctacccgatgatgcatctcgtttgtcatgggatgtcttagctgagcatggaaatatgttgtctgtatctctgctgtttgttttagagagattaagggcccaagttgcgagcgatggtgcggatggtgctccttccactgggatggcattttcatttgcacccggtgtgactgtagaagggttcctgtttgacgtggtaactacaggcgagtag

SEQ ID NO: 72 - DNA, 1173 bp, Synthetic construct
  source 1..1173: mol_type = other DNA
atgaataccactgaacaacaatcagtcttgcctcaacaagcttggctgggagcaccaccagcccctccaactagcgttgcagtcatagaatcactggctacatcaagccccactcaaacctatggccaagctgaatccgctgatcgtgttgccgcgagatttgatgaccctagacaggctgaacgtattagaagggtttacgctaaaactcgtgttacggaaaggcatttagccattgatccattgactcctgagtttgctgaatttagcgcaaggcctgatacagttagggaaagaatggatttattttttgaacacgcagcacccttagctatagaaacagcaagaagagccctaggcgataatgcggccactgatattggtcagctagtttttgtgacatctacgggctttcttgcacctggtgtagatgttgccgttatcagagccttaggtctagcgcctcaaacctccagagttgttattaatttcatgggatgtgccgctgcaatgaatgccttgagagttagtaccgattatgtgagagcacaacctgatagaaagtcactgatgatttgcttagaattgagttccgtcaatgccgtatttagcggtgaccctaacgatgttgtcattagttcattgttcgctgatggttgcggtgcagctgtaataggtgcttccgaagtcggccatccattgccttctggccagatcgttgtaagggatacgtttactcatttgttagatggtgcggaagatgggatagtgctgggcgtcaacgcaaatgggatcacttgtgaattagcagaaagccttccacagtacattgtcaacggggtagctcccgtagtcgacgcagttttggacaggaacgggttggggagggaggcagttgcacattgggctatccatcctggaggtcctaaaataatagaatcagcagcagctgctttaggtctacccgatgatgcatctcgtttgtcatgggatgtcttagctgagcatggaaatattttgtctgtatctctgctgtttgttttagagagattaagggcccaagttgcgagcgatggtgcggatggtgctccttccactgggatggcattttcatttgcacccggtgtgactgtagaagggttcctgtttgacgtggtaactacaggcgagtag

SEQ ID NO: 73 - DNA, 218 bp, Saccharomyces cerevisiae
  source 1..218: mol_type = genomic DNA
actcttttcttctaaccaagggggtggtttagtttagtagaacctcgtgaaacttacatttacatatatataaacttgcataaattggtcaatgcaagaaatacatatttggtcttttctaattcgtagtttttcaagttcttagatgctttctttttctcttttttacagatcatcaaggaagtaattatctactttttacaacaaatataaaacaa

SEQ ID NO: 74 - DNA, 673 bp, Saccharomyces cerevisiae
  source 1..673: mol_type = genomic DNA
agtttatcattatcaatactgccatttcaaagaatacgtaaataattaatagtagtgattttcctaactttatttagtcaaaaaattagccttttaattctgctgtaacccgtacatgcccaaaatagggggcgggttacacagaatatataacatcgtaggtgtctgggtgaacagtttattcctggcatccactaaatataatggagcccgctttttaagctggcatccagaaaaaaaaagaatcccagcaccaaaatattgttttcttcaccaaccatcagttcataggtccattctcttagcgcaactacagagaacaggggcacaaacaggcaaaaaacgggcacaacctcaatggagtgatgcaacctgcctggagtaaatgatgacacaaggcaattgacccacgcatgtatctatctcattttcttacaccttctattaccttctgctctctctgatttggaaaaagctgaaaaaaaaggttgaaaccagttccctgaaattattcccctacttgactaataagtatataaagacggtaggtattgattgtaattctgtaaatctatttcttaaacttcttaaattctacttttatagttagtcttttttttagttttaaaacaccaagaacttagtttcgaataaacacacataaacaaacaaa

SEQ ID NO: 75 - DNA, 450 bp, Saccharomyces cerevisiae
  source 1..450: mol_type = genomic DNA
ctacttattcccttcgagattatatctaggaacccatcaggttggtggaagattacccgttctaagacttttcagcttcctctattgatgttacacctggacaccccttttctggcatccagtttttaatcttcagtggcatgtgagattctccgaaattaattaaagcaatcacacaattctctcggataccacctcggttgaaactgacaggtggtttgttacgcatgctaatgcaaaggagcctatatacctttggctcggctgctgtaacagggaatataaagggcagcataatttaggagtttagtgaacttgcaacatttactattttcccttcttacgtaaatatttttctttttaattctaaatcaatctttttcaattttttgtttgtattcttttcttgcttaaatctataactacaaaaaacacatacataaactaaaa

SEQ ID NO: 76 - DNA, 331 bp, Saccharomyces cerevisiae
  source 1..331: mol_type = genomic DNA
gcccggtaccaagatggcctttggtgggttgaagaaggaaaaagacagaaacgacttaattacctacttgaaaaaagcctgtgagtaaacaggccccttttcctttgtcgatatcatgtaattagttatgtcacgcttacattcacgccctccccccacatccgctctaaccgaaaaggaaggagttagacaacctgaagtctaggtccctatttatttttttatagttatgttagtattaagaacgttatttatatttcaaatttttcttttttttctgtacagacgcgtgtacgcatgtaacattatactgaaaaccttgcttgagaag